European Patent Specification EP 3 517 631 B9, published October 4, 2023. Title: Mutant microorganisms to synthesize colanic acid, mannosylated and/or fucosylated oligosaccharides. Applicant: INBIOSE NV. The sequence listing filed with the application follows.

SEQUENCE LISTING (90 sequences)

SEQ ID NO: 1 - DNA, 3638 bp, Artificial sequence
  Vector
cgcgttggatgcaggcatgcaagcttggctgttttggcggatgagagaagattttcagcctgatacagattaaatcagaacgcagaagcggtctgataaaacagaatttgcctggcggcagtagcgcggtggtcccacctgaccccatgccgaactcagaagtgaaacgccgtagcgccgatggtagtgtggggtctccccatgcgagagtagggaactgccaggcatcaaataaaacgaaaggctcagtcgaaagactgggcctttcgttttatctgttgtttgtcggtgaacgctctcctgagtaggacaaatccgccgggagcggatttgaacgttgcgaagcaacggcccggagggtggcgggcaggacgcccgccataaactgccaggcatcaaattaagcagaaggccatcctgacggatggcctttttgcgtttctacaaactctttttgtttatttttctaaatacattcaaatatgtatccgctcatgagacaataaccctgataaatgcttcaataatattgaaaaaggaagagtatgagtattcaacatttccgtgtcgcccttattcccttttttgcggcattttgccttcctgtttttgctcacccagaaacgctggtgaaagtaaaagatgctgaagatcagttgggtgcacgagtgggttacatcgaactggatctcaacagcggtaagatccttgagagttttcgccccgaagaacgttttccaatgatgagcacttttaaagttctgctatgtggcgcggtattatcccgtgttgacgccgggcaagagcaactcggtcgccgcatacactattctcagaatgacttggttgagtactcaccagtcacagaaaagcatcttacggatggcatgacagtaagagaattatgcagtgctgccataaccatgagtgataacactgcggccaacttacttctgacaacgatcggaggaccgaaggagctaaccgcttttttgcacaacatgggggatcatgtaactcgccttgatcgttgggaaccggagctgaatgaagccataccaaacgacgagcgtgacaccacgatgcctacagcaatggcaacaacgttgcgcaaactattaactggcgaactacttactctagcttcccggcaacaattaatagactggatggaggcggataaagttgcaggaccacttctgcgctcggcccttccggctggctggtttattgctgataaatctggagccggtgagcgtgggtctcgcggtatcattgcagcactggggccagatggtaagccctcccgtatcgtagttatctacacgacggggagtcaggcaactatggatgaacgaaatagacagatcgctgagataggtgcctcactgattaagcattggtaactgtcagaccaagtttactcatatatactttagattgatttaaaacttcatttttaatttaaaaggatctaggtgaagatcctttttgataatctcatgaccaaaatcccttaacgtgagttttcgttccactgagcgtcagaccccgtagaaaagatcaaaggatcttcttgagatcctttttttctgcgcgtaatctgctgcttgcaaacaaaaaaaccaccgctaccagcggtggtttgtttgccggatcaagagctaccaactctttttccgaaggtaactggcttcagcagagcgcagataccaaatactgtccttctagtgtagccgtagttaggccaccacttcaagaactctgtagcaccgcctacatacctcgctctgctaatcctgttaccagtggctgctgccagtggcgataagtcgtgtcttaccgggttggactcaagacgatagttaccggataaggcgcagcggtcgggctgaacggggggttcgtgcacacagcccagcttggagcgaacgacctacaccgaactgagatacctacagcgtgagctatgagaaagcgccacgcttcccgaagggagaaaggcggacaggtatccggtaagcggcagggtcggaacaggagagcgcacgagggagcttccagggggaaacgcctggtatctttatagtcctgtcgggtttcgccacctctgacttgagcgtcgatttttgtgatgctcgtcaggggggcggagcctatggaaaaacgccagcaacgcggcctttttacggttcctggccttttgctggccttttgctcacatgttctttcctgcgttatcccctgattctgtggataaccgtattaccgcctttgagtgagctgataccgctcgccgcagccgaacgaccgagcgcagcgagtcagtgagcgaggaagcggaagagcgcctgatgcggtattttctccttacgcatctgtgcggtatttcacaccgcatatggtgcactctcagtacaatctgctctgatgccgcatagttaagccagtatacactccgctatcgctacgtgactgggtcatggctgcgccccgacacccgccaacacccgctgacgcgccctgacgggcttgtctgctcccggcatccgcttacagacaagctgtgaccgtctccgggagagctcgatatcccgggcggccgccttcattctataagtttcttgacatcttggccggcatatggtataatagggaaatttccatggcggccgctctagaagaagcttgggatccgtcgacctcgaattcggaggaaacaaagatggcctttaaagttgttcagatttgtggtggtctgggcaatcagatgtttcagtatgcatttgcaaaaagcctgcagaaacatagcaatacaccggttctgctggatattaccagctttgattggagcaatcgtaaaatgcagctggaactgtttccgattgatctgccgtatgcaagcgaaaaagaaattgcaattgccaaaatgcagcatctgccgaaactggttcgtaatgttctgaaatgcatgggttttgatcgtgtgagccaagaaatcgtgtttgaatatgaaccgaaactgctgaaaaccagccgtctgacctatttttatggctattttcaggatccgcgttattttgatgcaattagtccgctgatcaaacagacctttaccctgcctccgcctccggaaaatggtaataacaaaaaaaaagaagaagagtatcatcgtaaactggcactgattctggcagcaaaaaatagcgtgtttgtgcatattcgtcgcggtgattatgttggtattggttgtcagctgggcatcgattatcagaaaaaagcactggaatacatggcaaaacgtgttccgaatatggaactgtttgtgttttgcgaggacctggaatttacccagaatctggatctgggctatccgtttatggatatgaccacccgtgataaagaggaagaggcatattgggatatgctgctgatgcagagctgtaaacatggtattattgccaacagcacctatagttggtgggcagcatatctgattaataacccggaaaaaatcattattggtccgaaacattggctgtttggccatgaaaacatcctgtgtaaagaatgggtgaaaatcgaaagccactttgaagtgaaaagccagaaatataatgcctaataagagctcccaa

SEQ ID NO: 2 - DNA, 4311 bp, Artificial sequence
  Plasmid
aattcggaggaaacaaagatggggggttctcatcatcatcatcatcatggtatggctagcatgaaaaacaaggtgcagctcatcacttacgccgaccgccttggcgacggcaccatcaagtcgatgaccgacattctgcgcacccgcttcgacggcgtgtacgacggcgttcacatcctgccgttcttcaccccgttcgacggcgccgacgcaggcttcgacccgatcgaccacaccaaggtcgacgaacgtctcggcagctgggacgacgtcgccgaactctccaagacccacaacatcatggtcgacgccatcgtcaaccacatgagttgggaatccaagcagttccaggacgtgctggccaagggcgaggagtccgaatactatccgatgttcctcaccatgagctccgtgttcccgaacggcgccaccgaagaggacctggccggcatctaccgtccgcgtccgggcctgccgttcacccactacaagttcgccggcaagacccgcctcgtgtgggtcagcttcaccccgcagcaggtggacatcgacaccgattccgacaagggttgggaatacctcatgtcgattttcgaccagatggccgcctctcacgtcagctacatccgcctcgacgccgtcggctatggcgccaaggaagccggcaccagctgcttcatgaccccgaagaccttcaagctgatctcccgtctgcgtgaggaaggcgtcaagcgcggtctggaaatcctcatcgaagtgcactcctactacaagaagcaggtcgaaatcgcatccaaggtggaccgcgtctacgacttcgccctgcctccgctgctgctgcacgcgctgagcaccggccacgtcgagcccgtcgcccactggaccgacatacgcccgaacaacgccgtcaccgtgctcgatacgcacgacggcatcggcgtgatcgacatcggctccgaccagctcgaccgctcgctcaagggtctcgtgccggatgaggacgtggacaacctcgtcaacaccatccacgccaacacccacggcgaatcccaggcagccactggcgccgccgcatccaatctcgacctctaccaggtcaacagcacctactattcggcgctcgggtgcaacgaccagcactacatcgccgcccgcgcggtgcagttcttcctgccgggcgtgccgcaagtctactacgtcggcgcgctcgccggcaagaacgacatggagctgctgcgtaagacgaataacggccgcgacatcaatcgccattactactccaccgcggaaatcgacgagaacctcaagcgtccggtcgtcaaggccctgaacgcgctcgccaagttccgcaacgagctcgacgcgttcgacggcacgttctcgtacaccaccgatgacgacacgtccatcagcttcacctggcgcggcgaaaccagccaggccacgctgacgttcgagccgaagcgcggtctcggtgtggacaacgctacgccggtcgccatgttggaatgggaggattccgcgggagaccaccgttcggatgatctgatcgccaatccgcctgtcgtcgcctgactgcaggtcgaccatatgggagagctcccaacgcgttggatgcaggcatgcaagcttggctgttttggcggatgagagaagattttcagcctgatacagattaaatcagaacgcagaagcggtctgataaaacagaatttgcctggcggcagtagcgcggtggtcccacctgaccccatgccgaactcagaagtgaaacgccgtagcgccgatggtagtgtggggtctccccatgcgagagtagggaactgccaggcatcaaataaaacgaaaggctcagtcgaaagactgggcctttcgttttatctgttgtttgtcggtgaacgctctcctgagtaggacaaatccgccgggagcggatttgaacgttgcgaagcaacggcccggagggtggcgggcaggacgcccgccataaactgccaggcatcaaattaagcagaaggccatcctgacggatggcctttttgcgtttctacaaactctttttgtttatttttctaaatacattcaaatatgtatccgctcatgagacaataaccctgataaatgcttcaataatattgaaaaaggaagagtatgagtattcaacatttccgtgtcgcccttattcccttttttgcggcattttgccttcctgtttttgctcacccagaaacgctggtgaaagtaaaagatgctgaagatcagttgggtgcacgagtgggttacatcgaactggatctcaacagcggtaagatccttgagagttttcgccccgaagaacgttttccaatgatgagcacttttaaagttctgctatgtggcgcggtattatcccgtgttgacgccgggcaagagcaactcggtcgccgcatacactattctcagaatgacttggttgagtactcaccagtcacagaaaagcatcttacggatggcatgacagtaagagaattatgcagtgctgccataaccatgagtgataacactgcggccaacttacttctgacaacgatcggaggaccgaaggagctaaccgcttttttgcacaacatgggggatcatgtaactcgccttgatcgttgggaaccggagctgaatgaagccataccaaacgacgagcgtgacaccacgatgcctacagcaatggcaacaacgttgcgcaaactattaactggcgaactacttactctagcttcccggcaacaattaatagactggatggaggcggataaagttgcaggaccacttctgcgctcggcccttccggctggctggtttattgctgataaatctggagccggtgagcgtgggtctcgcggtatcattgcagcactggggccagatggtaagccctcccgtatcgtagttatctacacgacggggagtcaggcaactatggatgaacgaaatagacagatcgctgagataggtgcctcactgattaagcattggtaactgtcagaccaagtttactcatatatactttagattgatttaaaacttcatttttaatttaaaaggatctaggtgaagatcctttttgataatctcatgaccaaaatcccttaacgtgagttttcgttccactgagcgtcagaccccgtagaaaagatcaaaggatcttcttgagatcctttttttctgcgcgtaatctgctgcttgcaaacaaaaaaaccaccgctaccagcggtggtttgtttgccggatcaagagctaccaactctttttccgaaggtaactggcttcagcagagcgcagataccaaatactgtccttctagtgtagccgtagttaggccaccacttcaagaactctgtagcaccgcctacatacctcgctctgctaatcctgttaccagtggctgctgccagtggcgataagtcgtgtcttaccgggttggactcaagacgatagttaccggataaggcgcagcggtcgggctgaacggggggttcgtgcacacagcccagcttggagcgaacgacctacaccgaactgagatacctacagcgtgagctatgagaaagcgccacgcttcccgaagggagaaaggcggacaggtatccggtaagcggcagggtcggaacaggagagcgcacgagggagcttccagggggaaacgcctggtatctttatagtcctgtcgggtttcgccacctctgacttgagcgtcgatttttgtgatgctcgtcaggggggcggagcctatggaaaaacgccagcaacgcggcctttttacggttcctggccttttgctggccttttgctcacatgttctttcctgcgttatcccctgattctgtggataaccgtattaccgcctttgagtgagctgataccgctcgccgcagccgaacgaccgagcgcagcgagtcagtgagcgaggaagcggaagagcgcctgatgcggtattttctccttacgcatctgtgcggtatttcacaccgcatatggtgcactctcagtacaatctgctctgatgccgcatagttaagccagtatacactccgctatcgctacgtgactgggtcatggctgcgccccgacacccgccaacacccgctgacgcgccctgacgggcttgtctgctcccggcatccgcttacagacaagctgtgaccgtctccgggagagctcgatatcccgggcggccgcttcatttataaatttcttgacattttggaatagatgtgatataatgtgtacatatccatggcggccgctctagaagaagcttgggatccgtcgacctcg

SEQ ID NO: 3 - DNA, 340 bp, Artificial sequence
  Promotor
tgtttatttatcactttggcagagtaattatcctgtgcactattaatagcaatgtcgccatgcacatttaccttgcagttaattgaataaaaatttaactggcatcagtcctaaaaaaattgatttcatccgcaggctattgacagaataattcagactggtctttcaggcatccagacacgctaccgcccctggctttttagctaccaatacactgatttagtttaatttttcacaccctctcagcatgcagtcgttgatgagaaagggttattacggaaattaacttccgaatataaggtgacattatggtaattgaatattggctttccaataatgc

SEQ ID NO: 4 - DNA, 101 bp, Artificial sequence
  Promotor
cgaggtcgacggatcccaagcttcttctagagcggccgccatggaaatttccctattataccatatgccggccaagatgtcaagaaacttatagaatgaag

SEQ ID NO: 5 - DNA, 44 bp, Artificial sequence
  Promotor
taagtgtcattcaatatggtttttaggagtttctttaggttgac

SEQ ID NO: 6 - DNA, 485 bp, Artificial sequence
  Promotor
tgtttatttatcactttggcagagtaattatcctgtgcactattaatagcaatgtcgccatgcacatttaccttgcagttaattgaataaaaatttaactggcatcagtcctaaaaaaattgatttcatccgcaggctattgacagaataattcagactggtctttcaggcatccagacacgctaccgcccctggctttttagctaccaatacactgatttagtttaatttttcacaccctctcagcatgcagtcgttgatgagaaagggttattacggaaattaacttccgaatataaggtgacattatggtaattgaatattggctttccaataatgccgaggtcgacggatcccaagcttcttctagagcggccgccatggaaatttccctattataccatatgccggccaagatgtcaagaaacttatagaatgaagtaagtgtcattcaatatggtttttaggagtttctttaggttgac

SEQ ID NO: 7 - DNA, 74 bp, Artificial sequence
  Primer
cataatggatttccttacgcgaaatacgggcagacatggcctgcccggttattagtgtaggctggagctgcttc

SEQ ID NO: 8 - DNA, 71 bp, Artificial sequence
  Primer
gtatgttgtgtggaattgtgagcggataacaatttcacacaggaaacagctcatatgaatatcctccttag

SEQ ID NO: 9 - DNA, 18 bp, Artificial sequence
  Primer
gcggttggaataatagcg

SEQ ID NO: 10 - DNA, 20 bp, Artificial sequence
  Primer
caggtttcccgactggaaag

SEQ ID NO: 11 - DNA, 75 bp, Artificial sequence
  Primer
agaccgccggttttaagcagcgggaacatctctgaacatacatgtaaaacctgcagtgtaggctggagctgcttc

SEQ ID NO: 12 - DNA, 82 bp, Artificial sequence
  Primer
gtctggcagggacctgcacacggattgtgtgtgttccagagatgataaaaaaggagttagtccatatgaatatcctccttag

SEQ ID NO: 13 - DNA, 21 bp, Artificial sequence
  Primer
gcgaatatcgggaaatgcagg

SEQ ID NO: 14 - DNA, 22 bp, Artificial sequence
  Primer
cagagattgttttacctgctgg

SEQ ID NO: 15 - DNA, 70 bp, Artificial sequence
  Primer
catatttctgtcacactctttagtgattgataacaaaagaggtgccaggagtgtaggctggagctgcttc

SEQ ID NO: 16 - DNA, 70 bp, Artificial sequence
  Primer
taaaaacgtttaaccagcgactcccccgcttctcgcgggggagttttctgcatatgaatatcctccttag

SEQ ID NO: 17 - DNA, 18 bp, Artificial sequence
  Primer
gccacaggtgcaattatc

SEQ ID NO: 18 - DNA, 23 bp, Artificial sequence
  Primer
cattttcgaagtcgccgggtacg

SEQ ID NO: 19 - DNA, 70 bp, Artificial sequence
  Primer
ggcgctacaatcttccaaagtcacaattctcaaaatcagaagagtattgcgtgtaggctggagctgcttc

SEQ ID NO: 20 - DNA, 70 bp, Artificial sequence
  Primer
ggttgccggatgcggcgtgaacgccttatccggcctacatatcgacgatgcatatgaatatcctccttag

SEQ ID NO: 21 - DNA, 20 bp, Artificial sequence
  Primer
ggctcctccaacaccgttac

SEQ ID NO: 22 - DNA, 20 bp, Artificial sequence
  Primer
tacatatcggcatcgacctg

SEQ ID NO: 23 - DNA, 19 bp, Artificial sequence
  Primer
taccgccatttggcctgac

SEQ ID NO: 24 - DNA, 20 bp, Artificial sequence
  Primer
aaagtgcgctttgtccatgc

SEQ ID NO: 25 - DNA, 69 bp, Artificial sequence
  Primer
gacttccggcaacagatttcattttgcattccaaagttcagaggtagtcgtgtaggctggagctgcttc

SEQ ID NO: 26 - DNA, 69 bp, Artificial sequence
  Primer
gcttctgtcatcggtttcagggtaaaggaatctgcctttttccgaaatccatatgaatatcctccttag

SEQ ID NO: 27 - DNA, 21 bp, Artificial sequence
  Primer
tagcgtccctggaaaggtaac

SEQ ID NO: 28 - DNA, 20 bp, Artificial sequence
  Primer
tccctcatcatccgtcatag

SEQ ID NO: 29 - DNA, 71 bp, Artificial sequence
  Primer
cactttccgctgattcggtgccagactgaaatcagcctataggaggaaatggtgtaggctggagctgcttc

SEQ ID NO: 30 - DNA, 70 bp, Artificial sequence
  Primer
gttgccgacaggttggtgatgattcccccaatgctgggggaatgtttttgcatatgaatatcctccttag

SEQ ID NO: 31 - DNA, 79 bp, Artificial sequence
  Primer
ggttgaaaaataaaaacggcgctaaaaagcgccgttttttttgacggtggtaaagccgagtgtaggctggagctgcttc

SEQ ID NO: 32 - DNA, 76 bp, Artificial sequence
  Primer
ggtcagggacttttgtacttcctgtttcgatttagttggcaatttaggtagcaaaccatatgaatatcctccttag

SEQ ID NO: 33 - DNA, 22 bp, Artificial sequence
  Primer
ctgccgaaaatgaaagccagta

SEQ ID NO: 34 - DNA, 22 bp, Artificial sequence
  Primer
ggaaagtgcatcaagaacgcaa

SEQ ID NO: 35 - DNA, 71 bp, Artificial sequence
  Primer
ttgccactcaggtatgatgggcagaatattgcctctgcccgccagaaaaaggtgtaggctggagctgcttc

SEQ ID NO: 36 - DNA, 77 bp, Artificial sequence
  Primer
gttcaacattaactcatcggatcagttcagtaactattgcattagctaacaataaaacatatgaatatcctccttag

SEQ ID NO: 37 - DNA, 21 bp, Artificial sequence
  Primer
cggtggaatgagatcttgcga

SEQ ID NO: 38 - DNA, 20 bp, Artificial sequence
  Primer
acttgctcccgacacgctca

SEQ ID NO: 39 - DNA, 71 bp, Artificial sequence
  Primer
ttgccactcaggtatgatgggcagaatattgcctctgcccgccagaaaaagccgcttacagacaagctgtg

SEQ ID NO: 40 - DNA, 77 bp, Artificial sequence
  Primer
gttcaacattaactcatcggatcagttcagtaactattgcattagctaacaataaaaagccatgacccgggaattac

SEQ ID NO: 41 - DNA, 44 bp, Artificial sequence
  Primer
ctattgcattagctaacaataaaactttttctggcgggcagagg

SEQ ID NO: 42 - DNA, 48 bp, Artificial sequence
  Primer
cctctgcccgccagaaaaagttttattgttagctaatgcaatagttac

SEQ ID NO: 43 - DNA, 20 bp, Artificial sequence
  Primer
gccagcgcgataatcaccag

SEQ ID NO: 44 - DNA, 19 bp, Artificial sequence
  Primer
tgcgcctgaatgtggaatc

SEQ ID NO: 45 - DNA, 70 bp, Artificial sequence
  Primer
ttttgatatcgaaccagacgctccattcgcggatgtactcaaggtcgaacgtgtaggctggagctgcttc

SEQ ID NO: 46 - DNA, 70 bp, Artificial sequence
  Primer
tctatggtgcaacgcttttcagatatcaccatcatgtttgccggactatgcatatgaatatcctccttag

SEQ ID NO: 47 - DNA, 70 bp, Artificial sequence
  Primer
tcaatatgccgctttgttaacgaaacctttgaacaccgtcaggaaaacgattttgatatcgaaccagacg

SEQ ID NO: 48 - DNA, 70 bp, Artificial sequence
  Primer
tgacaaatctaaaaaagcgcgagcgagcgaaaaccaatgcatcgttaatctctatggtgcaacgcttttc

SEQ ID NO: 49 - DNA, 70 bp, Artificial sequence
  Primer
cgctttgttaacgaaacctttgaacaccgtcaggaaaacgattttgatatcgaaccagacgctccattcg

SEQ ID NO: 50 - DNA, 70 bp, Artificial sequence
  Primer
cagtcgtgtcatctgattacctggcggaaattaaactaagagagagctctgtgtaggctggagctgcttc

SEQ ID NO: 51 - DNA, 70 bp, Artificial sequence
  Primer
cgaattagcctgccagccctgtttttattagtgcattttgcgcgaggtcacatatgaatatcctccttag

SEQ ID NO: 52 - DNA, 20 bp, Artificial sequence
  Primer
agcgcaacaggcatctggtg

SEQ ID NO: 53 - DNA, 20 bp, Artificial sequence
  Primer
tatatcaggccagccatccc

SEQ ID NO: 54 - DNA, 69 bp, Artificial sequence
  Primer
gctgaacttgtaggcctgataagcgcagcgtatcaggcaatttttataatcttcatttaaatggcgcgc

SEQ ID NO: 55 - DNA, 69 bp, Artificial sequence
  Primer
gcgcaacgcaattaatgtgagttagctcactcattaggcaccccaggcttcgcctacctgtgacggaag

SEQ ID NO: 56 - DNA, 70 bp, Artificial sequence
  Primer
gcgcaacgcaattaatgtgagttagctcactcattaggcaccccaggcttgtgtaggctggagctgcttc

SEQ ID NO: 57 - DNA, 70 bp, Artificial sequence
  Primer
gctgaacttgtaggcctgataagcgcagcgtatcaggcaatttttataatcttaagcgacttcattcacc

SEQ ID NO: 58 - DNA, 68 bp, Artificial sequence
  Primer
cgacgcttgttcctgcgctttgttcatgccggatgcggctaatgtagatcgctgaacttgtaggcctg

SEQ ID NO: 59 - DNA, 69 bp, Artificial sequence
  Primer
cattaatgcagctggcacgacaggtttcccgactggaaagcgggcagtgagcgcaacgcaattaatgtg

SEQ ID NO: 60 - DNA, 69 bp, Artificial sequence; identical to SEQ ID NO: 25
  Primer

SEQ ID NO: 61 - DNA, 69 bp, Artificial sequence
  Primer
gcttctgtcatcggtttcagggtaaaggaatctgcctttttccgaaatcaagcttgcatgcctgcatcc

SEQ ID NO: 62 - DNA, 20 bp, Artificial sequence
  Primer
agaggctattcggctatgac

SEQ ID NO: 63 - DNA, 20 bp, Artificial sequence
  Primer
cgccatgttggaatgggagg

SEQ ID NO: 64 - DNA, 70 bp, Artificial sequence
  Primer
tgattgttatactatttgcacattcgttggatcacttcgatgtgcaagaagacttccggcaacagatttc

SEQ ID NO: 65 - DNA, 70 bp, Artificial sequence
  Primer
aattgcagaattcatgtaggcctgataagcgaagcgcatcaggcatttttgcttctgtcatcggtttcag

SEQ ID NO: 66 - DNA, 19 bp, Artificial sequence
  Primer
taccgccatttggcctgac

SEQ ID NO: 67 - DNA, 20 bp, Artificial sequence
  Primer
aaagtgcgctttgtccatgc

SEQ ID NO: 68 - DNA, 70 bp, Artificial sequence
  Primer
atcggcattgcccagaaggggccgtttatgttgccagacagcgctactgagtgtaggctggagctgcttc

SEQ ID NO: 69 - DNA, 70 bp, Artificial sequence
  Primer
attcgagcagatgatttactaaaaaagtttaacattatcaggagagcattaagcttgcatgcctgcatcc

SEQ ID NO: 70 - DNA, 68 bp, Artificial sequence
  Primer
aagccgttatagtgcctcagtttaaggatcggtcaactaatccttaactgatcggcattgcccagaag

SEQ ID NO: 71 - DNA, 77 bp, Artificial sequence
  Primer
ttgattttcataggttaagcaaatcatcaccgcactgactatactctcgtattcgagcagatgatttactaaaaaag

SEQ ID NO: 72 - DNA, 20 bp, Artificial sequence
  Primer
gcgtcaggcagtgttgtatc

SEQ ID NO: 73 - DNA, 20 bp, Artificial sequence
  Primer
ctggaagtgacgcattagag

SEQ ID NO: 74 - DNA, 22 bp, Artificial sequence
  Primer
tgtcattacttacacatcccgc

SEQ ID NO: 75 - DNA, 22 bp, Artificial sequence
  Primer
gcattcaatacgggtattgtgg

SEQ ID NO: 76 - DNA, 70 bp, Artificial sequence
  Primer
cattggggattatctgaatcagctcccctggaatgcaggggagcggcaaggtgtaggctggagctgcttc

SEQ ID NO: 77 - DNA, 70 bp, Artificial sequence
  Primer
tatttttagtagcttaaatgtgattcaacatcactggagaaagtcttatgaagcttgcatgcctgcatcc

SEQ ID NO: 78 - DNA, 72 bp, Artificial sequence
  Primer
caattacagtttctgactcaggactattttaagaatagaggatgaaaggtcattggggattatctgaatcag

SEQ ID NO: 79 - DNA, 80 bp, Artificial sequence
  Primer
gaatttttcaatatcgccatagctttcaattaaatttgaaattttgtaaaatatttttagtagcttaaatgtgattcaac

SEQ ID NO: 80 - DNA, 20 bp, Artificial sequence
  Primer
ttcaccgctaaagcggttac

SEQ ID NO: 81 - DNA, 20 bp, Artificial sequence
  Primer
cgcgtaatgcgtgggctttc

SEQ ID NO: 82 - DNA, 21 bp, Artificial sequence
  Primer
ccggcatatggtataataggg

SEQ ID NO: 83 - DNA, 18 bp, Artificial sequence
  Primer
acggcttgctggccatca

SEQ ID NO: 84 - DNA, 68 bp, Artificial sequence
  Primer
cgaatataaggtgacattatggtaattgaatattggctttccaataatgctacggccccaaggtccaa

SEQ ID NO: 85 - DNA, 70 bp, Artificial sequence
  Primer
aatattgtcaacctaaagaaactcctaaaaaccatattgaatgacacttattggcttcagggatgaggcg

SEQ ID NO: 86 - DNA, 20 bp, Artificial sequence
  Primer
tcccgactacgtggaccttg

SEQ ID NO: 87 - DNA, 90 bp, Artificial sequence
  Primer
catatggtataatagggaaatttccatggcggccgctctagaagaagcttgggatccgtcgacctcggcattattggaaagccaatattc

SEQ ID NO: 88 - DNA, 86 bp, Artificial sequence
  Primer
gccgccatggaaatttccctattataccatatgccggccaagatgtcaagaaacttatagaatgaagtaagtgtcattcaatatgg

SEQ ID NO: 89 - DNA, 73 bp, Artificial sequence
  Primer
aatattgtcaacctaaagaaactcctaaaaaccatattgaatgacacttacttcattctataagtttcttgac

SEQ ID NO: 90 - DNA, 74 bp, Artificial sequence
  Primer
cgaatataaggtgacattatggtaattgaatattggctttccaataatgccgaggtcgacggatcccaagcttc